European Patent Application EP 4 372 077 A1, published May 22, 2024. Title: COMPOSITION FOR IMPROVING AUTOPHAGY ACTIVATION. Applicant: MEIJI CO., LTD. The sequence listing filed with the application follows.

SEQUENCE LISTING (2 sequences)

SEQ ID NO: 1 - DNA, 533 bp, Lactobacillus plantarum
  source 1..533: mol_type = genomic DNA
ttaaagctggcggcgtgcctaatacatgcaagtcgaacgaactctggtattgattggtgcttgcatcatgatttacatttgagtgagtggcgaactggtgagtaacacgtgggaaacctgcccagaagcgggggataacacctggaaacagatgctaataccgcataacaacttggaccgcatggtccgagtttgaaagatggcttcggctatcacttttggatggtcccgcggcgtattagctagatggtggggtaacggctcaccatggcaatgatacgtagccgacctgagagggtaatcggccacattgggactgagacacggcccaaactcctacgggaggcagcagtagggaatcttccacaatggacgaaagtctgatggagcaacgccgcgtgagtgaagaagggtttcggctcgtaaaactctgttgttaaagaagaacatatctgagagtaactgttcaggtattgacggtatttaaccagaaagccacggctaactacgtgccagcagcccgcgggtctcta

SEQ ID NO: 2 - DNA, 445 bp, Lactobacillus farciminis
  source 1..445: mol_type = genomic DNA
tcatgattcagaccttggtgagtggcggacgggtgagtaacacgtgggtaacctgcccaaaagtgggggataacatttggaaacaagtgctaataccgcataacaactactttcacatgatcgtagcttgaaagatggctctgctatcgcttttggatggacccgcggcgtattagctagttggtgaggtaatagctcaccaaggcaatgatacgtagccgacctgagagggtaatcggccacattgggactgagacacggcccaaactcctacgggaggcagcagtagggaatcttccacaatgggcgaaagcctgatggagcaatgccgcgtgagtgaagaaggttttcggatcgtaaaactctgttgttgaagaagaacatgcgtgagagtaactgttcacgtactgacggtattcaaccagaaagccacggctaactacgt